European Patent Specification EP 3 630 960 B1, published December 13, 2023. Title: Method for preparing phosphorylated keto polyols, derivatives thereof, and uses thereof. Applicant: Commissariat à l'énergie atomique et aux énergies alternatives. The sequence listing filed with the application follows.

SEQUENCE LISTING (35 sequences)

SEQ ID NO: 1 - protein, 274 aa, Escherichia coli
MQNITQSWFVQGMIKATTDAWLKGWDERNGGNLTLRLDDADIAPYHDNFHQQPRYIPLSQPMPLLANTPFIVTGSGKFFRNVQLDPAANLGIVKVDSDGAGYHILWGLTNEAVPTSELPAHFLSHCERIKATNGKDRVIMHCHATNLIALTYVLENDTAVFTRQLWEGSTECLVVFPDGVGILPWMVPGTDEIGQATAQEMQKHSLVLWPFHGVFGSGPTLDETFGLIDTAEKSAQVLVKVYSMGGMKQTISREELIALGKRFGVTPLASALAL

SEQ ID NO: 2 - protein, 278 aa, Listeria welshimeri
MYSIYEAPFMKEMCEMTQNLWRNGWAEKNGGNISQLLEASEIKHYLDTDRYLWTEPLGFDASPLAGNVFLVSGSGKYFKNVQKNPADNLCIIKVSSDGASYHLLWGLENGGRPTSELASHLKCHIVRLSQDPDHRVILHTHATAVSAMTFVHDLDEAKFTRTLWQMITECLVVFPDGVAVVPWMVAGTNELGEASAAKMNDSRIVVWAHHGIMGAGTTMDDAFGLVETVEKAAKIYMQIAHFPTGIKQAITDEELVALAERFNVVPKAGILKEAGGVK

SEQ ID NO: 3 - protein, 270 aa, Clostridium hylemonae
MKNILESPIITEICDMTANMYRLGWDERNGGNISWLLDEQELAEYLDLSQVIRNIPIAFDAAELAGRIFLVTGTGKYFKNVTGNPQENLGIVRVASNGTELELLWGFEGGALPTSEFPTHLMNHMARLKADPEHRIVMHCHPANTIAMTFVHSIDDREFTCTLWQMITECIVVFPDGVGVVPWMVSGTNDIGEATARKIKDCRLVVWAHHGIFGTGRTLDEAFGLIETVEKAAQIYMKIAHLDIKNTIPKEQLKALAETFHAVPREGWLD

SEQ ID NO: 4 - protein, 296 aa, Lactobacillus rhamnosus
MDNKKQFLNPEYTQSFVESPYVAQMRKVTWNLYQHGWDERNGGNVSYRLTAAEIAPYGDVHEVKRNLPIKFDASELAGQYFLVTGTGRYFKNVKDFPARDTGLVQIAKDGHSVDLLWGFNDGGQPTSEFPSHLMTHIQRLKQDPNQRVVMHCHPTNLVAMSFTLPLEEKLFSRILWKMQAESIVVFPEGIGVLPYMTPGTNEIGQATAQKMADFRIVMWPQHGIFGAGDSIDETYGLIETVEKAATIYTAIQAQGGRIINEITDENLEQLAKRFDLTPNLAFLHGDSLISQVTLKV

SEQ ID NO: 5 - protein, 275 aa, Serratia odorifera
MQRILSSWFVQGMIKATGDMWLKGWDERNGGNISLRLTDDDVAPYRADFVAEPRCEELSQPAAELADCWFLVTGSGKFFRNVPLAPEESLVLLQVNHNGTAYHIHWGLSQGGLPTSELASHFQSHIVRMQLSNGQDRVIMHCHATNLIALSFVEKLESASFTRLLWEGSTECLVVFPDGIGIVPWMVPGTDGIGVKTAEQMRHHSLVLWPFHGIFGCGPTLDEAFGLIDTAEKSAEIMVKVIAMGGKRQTISTEQFIALAARFGVTPMSAALEVQ

SEQ ID NO: 6 - protein, 274 aa, Cronobacter turicensis
MQRILSSWFVQGMVKATSDMWLKGWDERNGGNVSLRLDAADVEPYRDEFYPAPRSVELSQPRTELAGCWFLVTGSGKFFRNVQLDPADTLVLLQITDDGMAYHIHWGLANGGLPTSELASHFQSHAVRKAVSADKDRVIMHCHATNLIALSFVLELDEARFTRLLWEGSTECLVVFPDGIGIVPWMVPGTDGIGSATSEQMKTHTLVLWPHHGIFGTGPTLDEAFGLIDTAEKSAEILVKVLSMGGMKQTITREELIALGERFGVTPHAGAIAL

SEQ ID NO: 7 - protein, 273 aa, Providencia rettgeri
MQDILTSWFVQGMIKATSDMWLKGWDERNGGNVSLRLTEDDVAPFKHTFHADPRYIETTEPVKELANQYFIVTGSGKFFRNVALDPADNLGLVRIDNEGQGYHIVWGFVNGAIPTSEFAAHFQSHITRMQATNGANRVIMHCHATNIIALSYVLPLDSASITRHLWEMSTECLVVFPDGIGVLPWMVPGTDGIGLETAEQMKQHGLVLWPFHGIFGSGPTLDDAFGLIDTAEKSAEILVKVLSMGGKKQTISTENLIALAKRFNVTPMSDALK

SEQ ID NO: 8 - protein, 275 aa, Marvinbryantia formatexigens
MKVLEAEFVREFIRMCDDGWKQGWHERNGGNLSYRIRKEEIDAMKEDFNPAGAWLEIGTSVPGLRGEYFLVTGSGKHFRNVAGKPEESIGIIEIDDSGEHYRICWGLQDQARPTSELPTHLMNHEVKKTATGGAHRVIYHAHPANLIALTFLLPLKDEVFTRELWEMATECPVVFPAGIGVVGWMVPGGREIAVATSKLMEQYDAVVWAHHGLFASGEDFDNTFGLMHTIEKSAEILVKVLSVRPDKLQTIQPQDFRNLAAEFKVTLPEKFLYEK

SEQ ID NO: 9 - protein, 272 aa, Mitsuokella multacida
MDIQDSKFMEGFKRLTADAFKKGWHERNGGNLTYRVKPEEVEAVKESLHEVKEWQPIGNTVPGLAGEYFLVTGSGKYMRNVSLAPEENVALIKIDEKGEQYGIVWGLVNGGRPTSELPTHLAAHELKKKMTDGRNRIIYHAHPTNLIALTFVLPLKDKEFTRELWEMATEDPVIFPEGIGVVPWMVPGGKEIADASVKLMEKYRVVVWAHHGLFVCGDDFDEAFGLMDTVEKASEICVKVLSMGGKKQTIPREGFIQLAKDFHIDLNTDLLD

SEQ ID NO: 10 - protein, 269 aa, Bacteroides thetaiotaomicron
MKSILENRPALAKEVNKVAEVAGYLWQKGWAERNGGNITVNITEFVDDEIRRMEPISEVKSIGVTLPYLKGCYFYCKGTNKRMRDLARWPMENGSVIRILDDCASYVIIADEAVAPTSELPSHLSVHNDLLSKNSPYKASVHTHPIELIAMTHCEKFLQKDVATNLLWSMIPETKAFCPRGLGIIPYKLPSSVELAEATIKELQDYDVVMWEKHGVFAVDCDAMQAFDQIDVLNKSALIYIAAKNMGFEPDGMSQEQMKEMSVAFNLPK

SEQ ID NO: 11 - protein, 274 aa, Shimwellia blattae
MQQILDAWFVQGMIKATSDAWLKGWDERNGGNLTLRLDEDDIAPYTADFHATPRYIPLSQPMPELAGTPFIVTGSGKFFRNVALETAANIGVVRVDRDGAGYHILWGLEGDALPTSELPAHFLSHCARIRATGGKDRVIMHCHATNLIALTYVLENDTNLITRKLWEGSTECLVVFPDGVGILPWMVPGTDDIGQTTAREMDKHALVLWPFHGVFGSGPTLDEAFGLIDTAEKSAEILVKVLSMGGMKQTISREELAALAARFGVTPLAGALAL

SEQ ID NO: 12 - protein, 281 aa, Enterococcus avium
MKLHEINQAPFIKEMCEATSQLWAYGWAERNGGNISYRLPQEEVQYYLDSDQVKRTIPLDFTVKSLAGELFLVSGSGKYFKNIQKNPADSLAIIRISAEGDRYELLWGLEGGDLPTSELASHLQCHEVRLAQDPEHRVILHTHATAISAMTFIHDLDEKKFSKTLWQMITECLVVFPDGVSVLPWMVAGTSQLGAASADKMQNSRIVIWPHHGIMGAGQTMDDAFGLVETAEKAAEIYLQICSAKQEIKQQITDQQLLDLAEKFHVKPKSGILLEEGLRSD

SEQ ID NO: 13 - protein, 270 aa, [Clostridium] termitidis
MKDILTAPFITEICKLTSNLYRLGWDERNGGNISYIVPEAEAAEYLDIKKAIRNIPMTFDGTSLAGRIFVVTGTGKYFKNVMDAPGINLGIIKVKEDGKSLDLLWGYEDGGRPTSELPAHLMTHIERLKADPNHRVVIHSHPTNTIAMTFVHELDERAFTRTLWQMCTECLVVFPDGVGVLPWMLCGNEEIGRVTAQKMKEFRVVVWGMHGIFGTGRDLDETFGLIETVEKAAEIYIKIMNMPIRQTITDDNLKVLAGAFGVTPRAGYLE

SEQ ID NO: 14 - protein, 304 aa, Lactobacillus shenzhenensis
MDMKKQFLNPEYAPAFVDSPYVTQMRKTTWNLYSHGWDERNGGNVSYRLTADEIKMYGDVHSVLRNIPIKFDASALKGDYFLVTGTGRYFKNVTDFPQRDLGLVRIADDGKSVDLVWGFNDGGQPTSEFPAHLMTHIQRLQHDANQRIVMHCHPTNLVAMTFTLPWNEKLFSRILWKMQAESIVVFPEGVGVLPYMTPGTNEIGAATAKKMGAYRVVLWPLHGVFGAGDSIDEVYGLIETVEKAATIYTAIKSQGGQFVNEITDDDLHKLAARFDLTPNKDFINGKSLAEVLNGAASKEPVGAR

SEQ ID NO: 15 - protein, 274 aa, Dickeya dadantii
MQSILSSWFVQGMVKATGDMWLKGWDERNGGNISLRLTTEDITPYESDFYPQPRHEALSQPMPELANGWFIVTGSGKFFRNVPLDPAENLVLLQVDANGAGYRIFWGLTAGGLPTSELAAHFQSHIVRIGVSGGRDRVIMHCHATNLIALSYVLELTSATFTRELWEGSTECLVVFPDGVGIVPWMVPGTDAIGTATAEQMHHHSLVLWPFHGIFGTGPSLDDAFGLIDTAEKSAEIMVKVRAMGGKKQTISTEELIALGTRFGVSPMASALKQ

SEQ ID NO: 16 - protein, 274 aa, Pectobacterium carotovorum
MQAILSSWFVQGMIKATSDMWLKGWDERNGGNVSLRLTAEDVTPYESDFYPQPRHEALSQPMPALADCWFIVTGSGKFFRNVQLDPADSLVVLQVDSDGKGYRIFWGLTNGGLPTSELASHFQSHIVRMGVTHGRDRVIMHCHATNLIALSYVLELDTATFTRELWEGSTECLVVFPDGVGIVPWMVPGTDAIGDATSEQMKRHSLVLWPFHGIFGTGPTLDEAFGLIDTAEKSAEVMVKVRSMGGKKQTISTEELIALGKRFGVTPLEAALRV

SEQ ID NO: 17 - protein, 274 aa, Obesumbacterium proteus
MQSIIDSWFVQGMIKATSDMWLKGWDERNGGNVSLRLLEEEVAPFRADFNSQPRCVELTQPATELANSWFLVTGSGKFFRNVQIAPQENLVLLQVSADGMAYHIHWGLTKGGLPTSELAAHFQSHIVRMQVTNGDNRVIMHCHATNLIALSYVHDLDNAKFTRLLWEGSTECLVVFPDGIGIVPWMVPGTDGIGTQTAEQMRQHGLVLWPFHGIFGSGPTLDDAFGLIDTAEKSAEIMVKVLSMGGKKQTISTQELIALAARFGVTPMAAALED

SEQ ID NO: 18 - protein, 275 aa, Hungatella hathewayi
MRVTDAEFVKGFIRLCDDGFKQNWHERNGGNLSYRIKPEEVESVKEELTDSNPWQPIGTSVPKLAGEYFMVTGSGKYFRNVILDPAANSCIIEVDEAGENYRICWGLVNGGRPTSELPSHLMNHEVKKEVTGGKHRVIYHAHPTNVIALTFVLPLEDKVFTRELWEMATECPVVFPDGVGVVGWMVPGGRDIAVATSELMKKYDVAVWAHHGLFASGEDFDLTFGLMHTVEKSAEILVKVLSIRPDKLQTITPQNFKDLAKDFKVTLPEEFLYEK

SEQ ID NO: 19 - protein, 272 aa, Megamonas hypermegale
MLITNAEFIQGFIRLTDDAFKKGWHERNGGNLSYRIKPEEIEEIKSELKAPTNWIPIGVSVPNLANEYFLVSGTGRYMRNIILKPKDNICIAKIDDKGENYAIVWGLEKGGRPTSEFPTHLMNHSIKKDLTNGQNHVIYHAHPTNIIALTFVLPLNDKEFTRELWEMATEDPVIFPEGIGVVPWMVPGGSEIAKATSELMKKYNIVVWAHHGMFCSGKDFDEAFGLMDTAEKAAEICVKVRSMGGKKQTITTQNFLDLAKDFKIDLNKTFLK

SEQ ID NO: 20 - protein, 269 aa, Prevotella oryzae
MKSILEGRPALKKEVDKIAEVAGYLWQKGWAERNGGNITVNITDLVDDEIKNMPAISEVKQIGVTLPHLKGTYFFCKGTGMRMRDLARWPMDNGSIIRILDDCASYVIIADNPVNPTSELPSHLMVHNHLIEKGSTFKASLHTHPIELIAMTHIRKFMGKDVLTKLLWSMIPETKAFCPKGLGIIPYELPSSVKLAEETVRQLDDYDVAMWEKHGVFAIDNDIMAAFDQVDVLNKSALIYIAAKNMGADPEGMSDAQMVEMTKAFNLPK

SEQ ID NO: 21 - protein, 236 aa, Thermotoga maritima
MRETIREIQKVAYWLAIKGLSEANAGNISVRLDERPEGYEVKSVNEYGFDYDGPEMYLLITATGSRMREVYEDDSKICLLHVLPGKHYEILHGNGKPTSEFPTHLMIHAKFKEMNPEKKAIVHTHPLNLLTLMNLEEFQELLPKMMKIHPEVLIFFPQGISVVEFEKPGSVELGLKTVEKSEGKDAVLWDKHGVVAFGKDVAEAYDRVEILEKAAEILLRVLSLGRNPTGVPEGWL

SEQ ID NO: 22 - protein, 215 aa, Escherichia coli
MERNKLARQIIDTCLEMTRLGLNQGTAGNVSVRYQDGMLITPTGIPYEKLTESHIVFIDGNGKHEEGKLPSSEWRFHMAAYQSRPDANAVVHNHAVHCTAVSILNRSIPAIHYMIAAAGGNSIPCAPYATFGTRELSEHVALALKNRKATLLQHHGLIACEVNLEKALWLAHEVEVLAQLYLTTLAITDPVPVLSDEEIAVVLEKFKTYGLRIEE

SEQ ID NO: 23 - protein, 216 aa, Kyrpidia tusciae
MPENIQELRNALLDAAHRLAARGLVPGTTGNVSLRIPGTDRFLITPTGIPYDVLHASDMVEVNLQGAVVEGNRKPSSETPLHTRIYHNHPWAGAVVHTHSMFATTFAVLNEAIPAVHYVIAGMGTDIPVAQYATYGSEDLAVNAAELISPEQRAILLQNHGVITVGGHLEEALHHAETVEYLAELYYRSRSIGSPNILPEEEIRRVAEKFKTYGQR

SEQ ID NO: 24 - protein, 516 aa, Acinetobacter baylyi
MLVLSACNDNHDNNSTSDRSATVETSAYVQTKTPYKPQQDLNTYQAAPTGFQPVFTELVARHGSRGLSSMKYDLALYNLWKQAKTENALTPLGEQLGADIEAIMKANILLGYGVAGIRQFGYGNESQLGIEEHRGIADRLLQRLPQLFNTSTLGQMDIAVQSSGVDRAVDSAKFFTNELIVKRPDLQEKIRPVSYASLSSDTYPSIDDQGVDRFLLYFHSLNKTTDLSQINSTLRQNIYDASLKYQDFEENDADLKQKLKELSSNNNAQQIALKVLTPLFKDEFIQKLGSQGYTFSNTGSFTTTASNGTQITEKGKGKNTIASTVDAAAYLYELYSIAPGMKKELGNTDFTKYMPIDAAKFYAEYNDAQDFYEKGPSFTESNQVTSNIANGLKQDFFAQVDQVINKQQQHKAVLRFAHAEIIIPLATAFELKGMMTPLALNQTYSYSTSTWRGEDISPMAANMQWDIYQNAQGYTLVKMLYNEKETLFKSSCDYARYNSSSFYYDYQKLKQCYGIN

SEQ ID NO: 25 - protein, 188 aa, Escherichia coli
MYERYAGLIFDMDGTILDTEPTHRKAWREVLGHYGLQYDIQAMIALNGSPTWRIAQAIIELNQADLDPHALAREKTEAVRSMLLDSVEPLPLVDVVKSWHGRRPMAVGTGSESAIAEALLAHLGLRHYFDAVVAADHVKHHKPAPDTFLLCAQRMGVQPTQCVVFEDADFGIQAARAAGMDAVDVRLL

SEQ ID NO: 26 - protein, 216 aa, Haemophilus influenzae
MNRAELSQKIIDTCLEMTKLGLNQGTAGNVSVRYKDGMLITPTGMPYHLMKTENIVYVDGNGKHEENKLPSSEWQFHLSVYHTRPEANAVVHNHSIHCAGLSILEKPIPAIHYMVAVSGTDHIPCVPYATFGSHKLASYVATGIKESKAILLAHHGLITCGENLDKALWLAQEVEVLASWYLKLLSTGLEIPLLSKEQMQVVLGKFHTYGLRIEES

SEQ ID NO: 27 - protein, 216 aa, Fusobacterium varium
MKLQTEREKVVKYLNLLIEKGLTKGTGGNISIYNEKENLVAISPSSVPYDILKPEDIMVVDLDGKVVDGNPMYVPSSETGMHLKVYKGREDIKALVHTHAMYCTTISCLREPLKAVDYMLAITGTNEVKCAEYAMFGTPELAENAFEAMRGAKACLLANHGVNVGAIDIENAFAITEYVEFCAELYVKARSIGNPVILSKEEIDRHIAKFGSYCKL

SEQ ID NO: 28 - protein, 221 aa, Brachyspira murdochii
MISQLNEYRKLLSNDIIKTCLRMQKDGINQGTSGNVSVRFENGMLITPSSMPYDTMKAENIVFVDENGKSEEGKRPSSEWRFHLSILKDNPDFNCVIHSHSIYSTVVSIMGVDYIPAIHYMIAVAGGKIIPCAEYATYGTEELCNNISKAMKGYKACIMKNHGLVVSDSTIEKAYGVLVEVENISREFVELSKIGKYNVLSDEDMDIILKKFGNYGLNAQK

SEQ ID NO: 29 - protein, 212 aa, Acetoanaerobium sticklandii
MMEYEKEQVVRYGKKLIDRRLTTGSGGNISVYNREQNLVAISPSGLDYYETTPEDIVILDIDGNLVEGKNRPSSEAGMHLAFYKNRADVSGIVHTHSKFATAIACMGWELPAVHYLIGMAGHRVKCTGYATYGSDELAKKALETIGDSNAVLLANHGLIALGEDVDRAFSTAEHLEFVSEVYYLTKTLGTPNILSDENMDEVMKKFGTFRYR

SEQ ID NO: 30 - protein, 226 aa, Blautia hydrogenotrophica
MLLQKERELVVEYGKKMSSSGLSKGTSGNISIYNRKEQLMAISPSGIGYFETMPEDVVIMDLHGNIVEGDKKPSSEWGLHTVFYLNKPDVEAVVHTHSTFCTTFACLNQPIRALHYVIGGAGTATVPCAPYRTFGTPELAEAAIEACGKGKAVLLANHGLLTCGPNIGKAFGLAVNMEFCAEMQFRAMCVGDPVILSDSEMENVMERFQSYGQPKKDGESKEPNCY

SEQ ID NO: 31 - protein, 213 aa, Enterococcus gilvus
MMEKEKELLVEYGKLLISTGLTTGTGGNISIYNPDEQIMAITPSGIDYFEMTVTDIVLLDLDGKVVEGKRKPSSEWQMHVINYQKRSDTIRAVVHAHSTFSSILATCRKSLPASNYMIAIAGGDDVRCSKYATFGTEELAEYAFEAMEDRYACFLANHGLLTGGFTLKEAFSVAVEIERLAGLHIGASLFGSPVILDESDMKKVQERFPSYGQ

SEQ ID NO: 32 - protein, 221 aa, Methylocella silvestris
MEKRGEFAVRQSIIDGCLALARLGVNQGTAGNISVRWNGGLLITPSGLPYDEMGADDIVFMAMDGSFRHPLAPSSEWRFHRDILARRPEVGAVVHAHPIFCTAFAMCRMEIPAAHYMIAAAGGPTIRCARYESYGTPELSEAALEALEGRACTLLANHGMIATGPDLAEALWLAVETETLARQYAAALQIGAPVILDDAEIAKTVEKFKDYGLRGRNRRDG

SEQ ID NO: 33 - protein, 217 aa, Roseobacter litoralis
MGQREDIITACKKLEADGLNRGASGNVSMRDGDHMLITPSAVGYDVIAPDMIARMRLDDDNGGWEGPNKPSSEWRFHRDILRGRPDINAVVHTHAPYATILAIARKPIPAVHYMIAAFGGPDIRVCDYARYGTAELSEHILEAMEGRNGCLMANHGMVVGASDLTRALWLAGELEALAHQYVHTLAIGGPVLLSDGEIEETAKGFESYGVQAKDTAQ

SEQ ID NO: 34 - protein, 218 aa, Rhodobacter sphaeroides
MNEMSDLSDLAKREEIIRQCLEMNRSGLNQGTSGNISVRHGEGMLITPTSLPYDTLVPEDIVFVSMEGEVRGRHKPSSEWRFHRDILRERADVNAVVHAHPTYCTTLAIMNREIPSIHYMLAVVGGPNIRCAPYAIYGSEELSRNAVEALHDRKACLLEHHGMIAVGKSLAQAMWLAVEVETLARQYHGCLQIGEPRLLSERQIQDVIDKIAGYGHQG

SEQ ID NO: 35 - protein, 286 aa, Escherichia coli
MSIISTKYLLQDAQANGYAVPAFNIHNAETIQAILEVCSEMRSPVILAGTPGTFKHIALEEIYALCSAYSTTYNMPLALHLDHHESLDDIRRKVHAGVRSAMIDGSHFPFAENVKLVKSVVDFCHSQDCSVEAELGRLGGVEDDMSVDAESAFLTDPQEAKRFVELTGVDSLAVAIGTAHGLYSKTPKIDFQRLAEIREVVDVPLVLHGASDVPDEFVRRTIELGVTKVNVATELKIAFAGAVKAWFAENPQGNDPRYYMRVGMDAMKEVVRNKINVCGSANRISA